European Patent Application EP 4 410 992 A1, published August 7, 2024. Title: METHODS FOR PRODUCING CLOSED LINEAR DNA. Applicant: 4basebio, S.L.U. Application EP. The sequence listing filed with the application follows.

SEQUENCE LISTING (32 sequences)

SEQ ID NO: 1 - DNA, 56 bp, synthetic construct
  source 1..56: mol_type = other DNA
tatcagcacacaattgcccattatacgcgcgtataatggactattgtgtgctgata

SEQ ID NO: 2 - DNA, 40 bp, synthetic construct
  source 1..40: mol_type = other DNA
cccattatacgcgcgtataatggactattgtgtgctgata

SEQ ID NO: 3 - DNA, 38 bp, synthetic construct
  source 1..38: mol_type = other DNA
cattatacgcgcgtataatggactattgtgtgctgata

SEQ ID NO: 4 - DNA, 36 bp, synthetic construct
  source 1..36: mol_type = other DNA
ttatacgcgcgtataatggactattgtgtgctgata

SEQ ID NO: 5 - DNA, 35 bp, synthetic construct
  source 1..35: mol_type = other DNA
tatacgcgcgtataatggactattgtgtgctgata

SEQ ID NO: 6 - DNA, 34 bp, synthetic construct
  source 1..34: mol_type = other DNA
atacgcgcgtataatggactattgtgtgctgata

SEQ ID NO: 7 - DNA, 37 bp, synthetic construct
  source 1..37: mol_type = other DNA
attatacgcgcgtataatggactattgtgtgctgata

SEQ ID NO: 8 - DNA, 21 bp, synthetic construct
  source 1..21: mol_type = other DNA
tatcagcacacaattgcccat

SEQ ID NO: 9 - DNA, 25 bp, synthetic construct
  source 1..25: mol_type = other DNA
atagtcgtgtgttaacgggtaatat

SEQ ID NO: 10 - DNA, 28 bp, synthetic construct
  source 1..28: mol_type = other DNA
atgttagtatcagcacacaattgcccat

SEQ ID NO: 11 - DNA, 32 bp, synthetic construct
  source 1..32: mol_type = other DNA
tacaatcatagtcgtgtgttaacgggtaatat

SEQ ID NO: 12 - DNA, 37 bp, synthetic construct
  source 1..37: mol_type = other DNA
ggccaacaaatgttagtatcagcacacaattgcccat

SEQ ID NO: 13 - DNA, 41 bp, synthetic construct
  source 1..41: mol_type = other DNA
ccggttgtttacaatcatagtcgtgtgttaacgggtaatat

SEQ ID NO: 14 - DNA, 20 bp, synthetic construct
  source 1..20: mol_type = other DNA
agggctaacatttgttggcc

SEQ ID NO: 15 - DNA, 16 bp, synthetic construct
  source 1..16: mol_type = other DNA
ggccaacaaatgttag

SEQ ID NO: 16 - DNA, 34 bp, synthetic construct
  source 1..34: mol_type = other DNA
ataacttcgtataatgtatgctatacgaagttat

SEQ ID NO: 17 - DNA, 40 bp, synthetic construct
  source 1..40: mol_type = other DNA
agggctaacatttgttggccactcaggccacaaatgttag

SEQ ID NO: 18 - DNA, 16 bp, synthetic construct
  source 1..16: mol_type = other DNA
ggccaacaaatgttag

SEQ ID NO: 19 - DNA, 20 bp, synthetic construct
  source 1..20: mol_type = other DNA
agggctaacatttgttggcc

SEQ ID NO: 20 - DNA, 33 bp, synthetic construct
  source 1..33: mol_type = other DNA
tacgcgcgtataatggactattgtgtgctgata

SEQ ID NO: 21 - DNA, 28 bp, synthetic construct
  source 1..28: mol_type = other DNA
tatcagcacacaattgcccattatacgc

SEQ ID NO: 22 - DNA, 28 bp, synthetic construct
  source 1..28: mol_type = other DNA
gcgtataatggactattgtgtgctgata

SEQ ID NO: 23 - DNA, 36 bp, synthetic construct
  source 1..36: mol_type = other DNA
tatcagcacacaattgcccattatacgcgcgtataa

SEQ ID NO: 24 - DNA, 25 bp, synthetic construct
  source 1..25: mol_type = other DNA
tataatggactattgtgtgctgata

SEQ ID NO: 25 - DNA, 21 bp, synthetic construct
  source 1..21: mol_type = other DNA
tacctgataacacacgactat

SEQ ID NO: 26 - DNA, 32 bp, synthetic construct
  source 1..32: mol_type = other DNA
tataatggactattgtgtgctgatactaacat

SEQ ID NO: 27 - DNA, 28 bp, synthetic construct
  source 1..28: mol_type = other DNA
tacctgataacacacgactatgattgta

SEQ ID NO: 28 - DNA, 41 bp, synthetic construct
  source 1..41: mol_type = other DNA
tataatggactattgtgtgctgatactaacatttgttggcc

SEQ ID NO: 29 - DNA, 37 bp, synthetic construct
  source 1..37: mol_type = other DNA
tacctgataacacacgactatgattgtaaacaaccgg

SEQ ID NO: 30 - DNA, 35 bp, synthetic construct
  source 1..35: mol_type = other DNA
tatcagcacacaattgcccattatacgcgcgtata

SEQ ID NO: 31 - DNA, 34 bp, synthetic construct
  source 1..34: mol_type = other DNA
tatcagcacacaattgcccattatacgcgcgtat

SEQ ID NO: 32 - DNA, 33 bp, synthetic construct
  source 1..33: mol_type = other DNA
tatcagcacacaattgcccattatacgcgcgta